European Patent Specification EP 3 097 911 B1, published May 22, 2024. Title: Metabolism improving agent comprising rare fatty acids. Applicant: Kyoto University Nitto Pharmaceutical Industries, Ltd. The sequence listing filed with the application follows.

SEQUENCE LISTING (2 sequences)

SEQ ID NO: 1 - DNA, 1773 bp, Lactobacillus acidophilus
  CDS (1)..(1773)
atgcattatagtagtggtaattatgaagcttttgtaaacgcaagtaaacctaaggatgtcgatcagaagtccgcatatcttgttggttcaggtttggcatcgcttgctagtgctgtatttttaattcgtgatggtcacatgaagggtgatagaattcatatccttgaagaattgagccttccaggtggttcaatggatgggatctataataagcaaaaagaaagctacatcattcgtggtggtcgtgaaatggaagcccattttgaatgcttgtgggacttgtttagatcgattccatcagctgaaaataaagatgaatcggtcctggatgaattttaccgtttaaatagaaaagatccaagtttcgcaaagactcgtgtcattgttaaccgcggacatgaacttccaactgacggtcaattacttcttactcccaaggctgttaaagaaattattgatctttgcttaactcctgaaaaagatttacaaaataaaaaaattaatgaagtctttagtaaagaattttttgaatcaaacttctggctttactggtcaacgatgtttgcctttgagccatgggcaagtgcgatggaaatgcgtcgttacttaatgcgttttgttcaacacgtttctacacttaagaatttatcatcactacgctttactaagtataaccaatatgaatcattaattttaccaatggttaaatacttgaaagatcgcggcgtgcaattccattacaacaccgttgttgataatatctttgttaaccgttcaaatggtgaaaagattgctaagcaaattcttttaactgaaaacggtgaaaaaaagagcatcgatttaacagaaaatgacctcgtcttcgttactaacggttcaattactgaaagtacaacttatggtgataacttgcacccagcttctgaggaacataaattaggtgctacttggaaattatggcaaaacttggcagcgcaagatgatgacttcggtcacccagatgtcttctgcaaggatattccaaaggctaactgggtaatgtctgctacaattacttttaagaataatgatattgtgccattcattgaagcagttaataagaaggatccacacagcggctcaattgtaactagtgggcctactacgattaaggattctaactggctacttggttattcaatcagtcgtcagcctcactttgaagcacaaaagcctaacgaattgattgtatggctttatggtttgttctcagacaccaaaggtaactatgttgaaaagactatgcctgactgtaacggtattgaattatgtgaagaatggctttaccacatgggtgttcctgaagaaagaatcccagaaatggcttcagctgctacgactattccagcacacatgccatatattacttcatacttcatgccaagagcattaggcgacagacccaaggttgtgccagaccactcaaagaacttggccttcattggtaactttgctgaaacgccaagagacactgtctttaccactgaatactctgtcagaactgcgatggaagctgtatacaccttgcttaacattgatcgtggtgtgccagaagtatttgcatctgccttcgatgtcagaatgctcatgaacgcaatgtactacttgaatgatcaaaagaagcttgaagatcttgatttgcctattgctgaaaagttggcaattaaggggatgctcaagaaagttaagggcacttatatagaggaattgcttaagaagtataagttggtttag

SEQ ID NO: 2 - protein, 590 aa, Lactobacillus acidophilus
MHYSSGNYEAFVNASKPKDVDQKSAYLVGSGLASLASAVFLIRDGHMKGDRIHILEELSLPGGSMDGIYNKQKESYIIRGGREMEAHFECLWDLFRSIPSAENKDESVLDEFYRLNRKDPSFAKTRVIVNRGHELPTDGQLLLTPKAVKEIIDLCLTPEKDLQNKKINEVFSKEFFESNFWLYWSTMFAFEPWASAMEMRRYLMRFVQHVSTLKNLSSLRFTKYNQYESLILPMVKYLKDRGVQFHYNTVVDNIFVNRSNGEKIAKQILLTENGEKKSIDLTENDLVFVTNGSITESTTYGDNLHPASEEHKLGATWKLWQNLAAQDDDFGHPDVFCKDIPKANWVMSATITFKNNDIVPFIEAVNKKDPHSGSIVTSGPTTIKDSNWLLGYSISRQPHFEAQKPNELIVWLYGLFSDTKGNYVEKTMPDCNGIELCEEWLYHMGVPEERIPEMASAATTIPAHMPYITSYFMPRALGDRPKVVPDHSKNLAFIGNFAETPRDTVFTTEYSVRTAMEAVYTLLNIDRGVPEVFASAFDVRMLMNAMYYLNDQKKLEDLDLPIAEKLAIKGMLKKVKGTYIEELLKKYKLV